European Patent Specification EP 3 784 348 B1, published August 5, 2026. Title: Method of Treatment. Applicant: The University Court of the University of Edinburgh. The sequence listing filed with the application follows.

SEQUENCE LISTING (18 sequences)

SEQ ID NO: 1 - RNA, 99 nt, Artificial Sequence
  miR-148b mimic corresponding to human precursor miR-148b
caagcacgauuagcauuugaggugaaguucuguuauacacucaggcuguggcucucugaaagucagugcaucacagaacuuugucucgaaagcuuucua

SEQ ID NO: 2 - RNA, 22 nt, Artificial Sequence
  mature hsa-miR-148b-5p
aaguucuguuauacacucaggc

SEQ ID NO: 3 - RNA, 22 nt, Artificial Sequence
  mature hsa-miR-148b-3p
ucagugcaucacagaacuuugu

SEQ ID NO: 4 - RNA, 7 nt, Artificial Sequence
  mature hsa-miR-148b-3p seed region sequence
cagugca

SEQ ID NO: 5 - RNA, 7 nt, Artificial Sequence
  mature hsa-miR-148b-5p seed region sequence
aguucug

SEQ ID NO: 6 - DNA, 20 bp, Artificial Sequence
  hsa-miR-148b-3p miRCURY lock nucleic acid (LNA)  miRNA Inhibitor (YI04101119) sequence
caaagttctgtgatgcactg

SEQ ID NO: 7 - DNA, 29 bp, Artificial Sequence
  TGFbeta2 3'UTR Forward Primer
ataaagcttatttgccacatcattgcaga

SEQ ID NO: 8 - DNA, 29 bp, Artificial Sequence
  TGFbeta2 3'UTR Reverse Primer
ataactagtgggaataaaaagacggcaca

SEQ ID NO: 9 - DNA, 34 bp, Artificial Sequence
  SMAD2 3'UTR Forward Primer
ataaagctttgatccagctaaggtaactgatgtt

SEQ ID NO: 10 - DNA, 34 bp, Artificial Sequence; identical to SEQ ID NO: 9
  SMAD2 3'UTR Reverse Primer

SEQ ID NO: 11 - DNA, 29 bp, Artificial Sequence
  TGFB2 3'UTR mutation forward primer
ataaagcttatttgccacatcattgcaga

SEQ ID NO: 12 - DNA, 33 bp, Artificial Sequence
  TGFB2 3'UTR mutation reverse primer
ataactagtcctatctgagaggaaaatgtctgc

SEQ ID NO: 13 - DNA, 34 bp, Artificial Sequence; identical to SEQ ID NO: 9
  SMAD2 3'UTR mutation forward primer

SEQ ID NO: 14 - DNA, 29 bp, Artificial Sequence
  SMAD2 3'UTR mutation reverse primer
ataactagtggacttccagagggaaacaa

SEQ ID NO: 15 - RNA, 23 nt, Homo sapiens
gucuuuccucaugaaugcacuga

SEQ ID NO: 16 - RNA, 22 nt, Artificial Sequence
  hsa-miR-148a-3p
uguuucaagacaucacgugacu

SEQ ID NO: 17 - RNA, 23 nt, Homo sapiens
uggcugcauccuuggugcacugu

SEQ ID NO: 18 - RNA, 22 nt, Artificial Sequence
  hsa-miR-148b-3p
uguuucaagacacuacgugacu